European Patent Application EP 4 183 799 A1, published May 24, 2023. Title: METHOD FOR PRODUCING ANTIBODY-DRUG CONJUGATE. Applicant: DAIICHI SANKYO COMPANY, LIMITED. The sequence listing filed with the application follows.

SEQUENCE LISTING (16 sequences)

SEQ ID NO: 1 - protein, 470 aa, Artificial Sequence
  Heavy chain of anti-TROP2 antibody
MKHLWFFLLLVAAPRWVLSQVQLVQSGAEVKKPGASVKVSCKASGYTFTTAGMQWVRQAPGQGLEWMGWINTHSGVPKYAEDFKGRVTISADTSTSTAYLQLSSLKSEDTAVYYCARSGFGSSYWYFDVWGQGTLVTVSSASTKGPSVFPLAPSSKSTSGGTAALGCLVKDYFPEPVTVSWNSGALTSGVHTFPAVLQSSGLYSLSSVVTVPSSSLGTQTYICNVNHKPSNTKVDKRVEPKSCDKTHTCPPCPAPELLGGPSVFLFPPKPKDTLMISRTPEVTCVVVDVSHEDPEVKFNWYVDGVEVHNAKTKPREEQYNSTYRVVSVLTVLHQDWLNGKEYKCKVSNKALPAPIEKTISKAKGQPREPQVYTLPPSREEMTKNQVSLTCLVKGFYPSDIAVEWESNGQPENNYKTTPPVLDSDGSFFLYSKLTVDKSRWQQGNVFSCSVMHEALHNHYTQKSLSLSPGK

SEQ ID NO: 2 - protein, 234 aa, Artificial Sequence
  Light chain of anti-TROP2 antibody
MVLQTQVFISLLLWISGAYGDIQMTQSPSSLSASVGDRVTITCKASQDVSTAVAWYQQKPGKAPKLLIYSASYRYTGVPSRFSGSGSGTDFTLTISSLQPEDFAVYYCQQHYITPLTFGQGTKLEIKRTVAAPSVFIFPPSDEQLKSGTASVVCLLNNFYPREAKVQWKVDNALQSGNSQESVTEQDSKDSTYSLSSTLTLSKADYEKHKVYACEVTHQGLSSPVTKSFNRGEC

SEQ ID NO: 3 - protein, 471 aa, Artificial Sequence
  Heavy chain of anti-B7-H3 antibody
MKHLWFFLLLVAAPRWVLSQVQLVQSGAEVKKPGSSVKVSCKASGYTFTNYVMHWVRQAPGQGLEWMGYINPYNDDVKYNEKFKGRVTITADESTSTAYMELSSLRSEDTAVYYCARWGYYGSPLYYFDYWGQGTLVTVSSASTKGPSVFPLAPSSKSTSGGTAALGCLVKDYFPEPVTVSWNSGALTSGVHTFPAVLQSSGLYSLSSVVTVPSSSLGTQTYICNVNHKPSNTKVDKRVEPKSCDKTHTCPPCPAPELLGGPSVFLFPPKPKDTLMISRTPEVTCVVVDVSHEDPEVKFNWYVDGVEVHNAKTKPREEQYNSTYRVVSVLTVLHQDWLNGKEYKCKVSNKALPAPIEKTISKAKGQPREPQVYTLPPSREEMTKNQVSLTCLVKGFYPSDIAVEWESNGQPENNYKTTPPVLDSDGSFFLYSKLTVDKSRWQQGNVFSCSVMHEALHNHYTQKSLSLSPGK

SEQ ID NO: 4 - protein, 233 aa, Artificial Sequence
  Light chain of anti-B7-H3 antibody
MVLQTQVFISLLLWISGAYGEIVLTQSPATLSLSPGERATLSCRASSRLIYMHWYQQKPGQAPRPLIYATSNLASGIPARFSGSGSGTDFTLTISSLEPEDFAVYYCQQWNSNPPTFGQGTKVEIKRTVAAPSVFIFPPSDEQLKSGTASVVCLLNNFYPREAKVQWKVDNALQSGNSQESVTEQDSKDSTYSLSSTLTLSKADYEKHKVYACEVTHQGLSSPVTKSFNRGEC

SEQ ID NO: 5 - protein, 5 aa, Artificial Sequence
  CDRH1 of anti-TROP2 antibody
TAGMQ

SEQ ID NO: 6 - protein, 17 aa, Artificial Sequence
  CDRH2 of anti-TROP2 antibody
WINTHSGVPKYAEDFKG

SEQ ID NO: 7 - protein, 12 aa, Artificial Sequence
  CDRH3 of anti-TROP2 antibody
SGFGSSYWYFDV

SEQ ID NO: 8 - protein, 11 aa, Artificial Sequence
  CDRL1 of anti-TROP2 antibody
KASQDVSTAVA

SEQ ID NO: 9 - protein, 7 aa, Artificial Sequence
  CDRL2 of anti-TROP2 antibody
SASYRYT

SEQ ID NO: 10 - protein, 9 aa, Artificial Sequence
  CDRL3 of anti-TROP2 antibody
QQHYITPLT

SEQ ID NO: 11 - protein, 5 aa, Artificial Sequence
  CDRH1 of anti-B7-H3 antibody
NYVMH

SEQ ID NO: 12 - protein, 17 aa, Artificial Sequence
  CDRH2 of anti-B7-H3 antibody
YINPYNDDVKYNEKFKG

SEQ ID NO: 13 - protein, 13 aa, Artificial Sequence
  CDRH3 of anti-B7-H3 antibody
WGYYGSPLYYFDY

SEQ ID NO: 14 - protein, 10 aa, Artificial Sequence
  CDRL1 of anti-B7-H3 antibody
RASSRLIYMH

SEQ ID NO: 15 - protein, 7 aa, Artificial Sequence
  CDRL2 of anti-B7-H3 antibody
ATSNLAS

SEQ ID NO: 16 - protein, 9 aa, Artificial Sequence
  CDRL3 of anti-B7-H3 antibody
QQWNSNPPT